European Patent Specification EP 3 837 368 B1, published January 11, 2023. Title: TRANSCRIPTIONAL REGULATORY ELEMENT AND ITS USE IN ENHANCING THE EXPRESSION OF EXOGENOUS PROTEIN. Applicant: WuXi Biologics （shanghai）Co., Ltd. The sequence listing filed with the application follows.

SEQUENCE LISTING (23 sequences)

SEQ ID NO: 1 - DNA, 27 bp, Artificial Sequence
gcaaaaaagggaataagggcgacacgg

SEQ ID NO: 2 - DNA, 28 bp, Artificial Sequence
catagcccatatatggagttccgcgtta

SEQ ID NO: 3 - DNA, 3619 bp, Chinese hamster
gatctgcctgcctctgccccgtgagtgctgggattaaaggccagcaccgccatgcctggcctcctttaagtgcaggtgtagcacgccagaaataccctgctggtgacagtgtgagccacatgcgtgagactgctgcagaggtcccagcttaggttgtgcccttctttcttgagaaatgtcttacttggtgattttgagtggaaacatgtatttagctgacatatgagcctagtcttttatgtataaatgtgtgttatatttctagatacaaaaatattaaaaattagaaatcttcagggctggagaggggttcattggttaagagctcattggttaagggctgctcctgtataggacccgggttacctgtcagcaccgtatgacggctctcaaccatctgcagctcccgttccagaggacccagtgtcttcttctggcctctacagacatacatatagacaaaacacccatacacaaaaatttaattagaaatcttaatttttttctttcaattttctagattgactggggataacttttttgttaactttactgtcttgaggataacgttcagtatgagttgtatttctagagtttgtctttatttttaggcaaaaataacctttattaccattttggggggtgactgttttacaacttttccaactttctgcttcatctcttgtgtcctatataggcccctatttactgtcattattagagataggacttgatgtcatgtcaactccatctttgttataaatctcaagaagagctaatttcttttgtgttattacaaccaaaaataaacaaggtagcttataaacagtgacttatttttatagttctagatatgggaagatcatggtgacagtagattcaatgtctagttggaagttgactcttcttcatagatggaatccttgctataatataatctcaggatggaagggatgagctaagccctctgggatctcttattaatctgttcattcatttacttattgcatagtgctctaattctgttcatggagactctgttcttacacattaggtggttagggagggacatgatcaatcaggacataggagcaacaataatttttattatatttcccaaaatacatggcagttcctgaccttgctttattactgcaaacatacagcttgtggccattggacttagccatatgagaaatgtaagaatttattttatattgtagctgcaaatggtaggttcatcaaattgtgccttaagttcacatcttaatttgctacaaaaaaaaaagaggagtagtgtaagttacatttaattttcaattacttagtaacagtttgtaagtgctacttgatcctgttttatatctagcattgagtatagatcaacaagtgtttcaattcttgtttggacatgctgttctctccttcatcacaagttacttctggctaaacaaggcacaaatttcgcatgaccaccaatccaaggacagggcgacaattttaatgagtttcattgagagctggccaactgagcatctgttccttttgttttcctgtacgtggtaagccagtgtttctacactccttagccttgttgctgtgtgtatagtgtggggtggatttgtttttgctgttcttttttcttttttctaccctctacttcagtggtgcacggttagaaatcttgtggcgtctggcacggtggtataattccttccatgctcttgggtgaggaaataagtttgctcattgctgctcatcagtctgtttcacttgctcccagatggtgaccttctcgtcccattcttgcttgttttaacattattctgacacctattttctttcattgtccccttaaccactctaattgaataatgatttctgtaatttccatttggaacacaaccagcttcctggttccttttattggcccacatcctgtcttctagttcattgcttcagatttgagccaaatcatcaaataaaaatacgtaactgaaaaaaatgtttattgcagtggcctcctctagcatggcaacaatgagagttttcctttcttattgctaaacatgttatatctgtctcatgatttcatactgtctctcctggcctcatttactgcttgacctttaaaagaaatgactcaaagatatttttgtagttctgtaagcatttctctagttcttgttcttcacctttagttcttaacagtagttttgtctgctacactgacgtggctgtgaggactttccttcagaaactggcgtctgatactgattcaaactggtctccattgtggcctacatgtccagctgtctccatgtaacgccactgaaatacagtgaagccagcctttttttcccccttatggttcaaagcaactgaatttcagtcagagtaattttggtttgggtatcaatactaattgtagtcttagaccttttaattattacttgtttgcattttacagaagacattggtccttctcaaaagcagagatgaaacctgtagtattttgtgtgtagttttcctctgctggttgccctgtaactattcagttcctgtaaggaagcacagctgcttcataagctaccttaggctgacagcagtctcctgaaagaaagagttcaagaaagaaacatttaaaaataaaaatggggaggggtccaagtagtatttgaagccatgaaatatcttgaatatagtttgcttttttgttttgttttgtctgtctgtctgtccgatgtagctttggccatatcaaccaggctgtccttgaactcacagaaatccacctgcctccgcctcccaagtgctggatgcaccaccatgccagctagtttgctttttagagcatctcatctgctgctcacagccctggtgctttatgggatttgtttggggaacatgatgagctctatatttattgtagctttaaatggacagcggttattgactgtcagcttagtctttaaaatctataatcacattgtacctaattgtcaaccttcatgttttttaattatgaaaaaaactgagaacattaatttttatgttatcttgttattgactttattgaaatactacagaaaattttggtttgaggcttttccataatttacccttacacctcacaccccttccataaacatgtgcagttaaaattgaattgttcgggcacttctaccttgatacctggcctacagtgggaaaggtctgtctttctttggaataagcccatcagtggccttgtgtacattctgtatttttgttgtttgttattactgttttttacttgggactaataatctgtttgaaactgactgagatagaaagatgtgatgttccttcccactcactccggattttgatagaagacttgttttatttatttccaaaattatatccgcaggaaacaagctgtttaaattcagattatgctgaagcaaaatggtcctggtatgagaagcaacgtgctgttttacgagcacagagtcccttttctcataactgattgatagtaaatattttcctgaagaattattgccaaccatgaacagtgcaactgtttcactttttttccgtgctacttgctgtaccagccattgtcggtaattaa

SEQ ID NO: 4 - DNA, 1114 bp, Chinese hamster
gatctgaagtttggatctgcagaacccacacaaaggcctacgggcttagtagtgtacctgcaatttcagcacttggaaggctgagaaaggatcccaagggcagctggctagctaggctagtgttagctgagagctctgggttcgtggagcgactctggttcagtgaataagatagagagtgacatcagctttgggcttccacagcaaatgagctcacttgcatgcaaacagaaatgcaaacacatgcacaaagcaaaacaaaaggaacacaggccaaaggtgggtcattcctataccatcccctcagcagggtgcagtccccacaccctgacccagttccctcatgatgttagagaaaataactttgcccccttcaacgaacatttcagctccagagaacctggcccactttgaaagctttaattagaaatgtgcaattacccggaacagatgtctgttgtgattgtggagacataggttaaagaatcacacagcagtttgcgtggttacagaaaggttgcaagtaactttaaaacacagtttttggtaagtctccaacatgttacctaacatagcatggcctcgattacatgtaagcagtgagtctccggctgcctggtttgtgagggtaatgtacttcagcaatagtgctgaggctgtacagtgagtgactcatcaccctaaaaaagtatcgaattccagtcttcagagttagctttcagtaaaaccaagtcagtggtgaaatggctcagtaggtaagggcacccgctgccaagcccaagacctgtgtcctgtccctgggatccagttggtggaaagagagaacggactcctgcaaggtggcctctgacctacatgcctgaattctgccagacattaagtaaaaacaaacgcaaaaagggaagtgggctcacgcataaggcactcactggactctactcttctactctgtggttactttttggtgttcaagcataccataccttgatctacatgatttttactccaaagacacagccagggtaatgttgtgtgatggatcagtcttatttgttacttgtttactagtacttactgagattgtcgatggctttaatgtcaacatgagtgtgga

SEQ ID NO: 5 - DNA, 4068 bp, Chinese hamster
gatcttctaggtctggctctgagttgaaaggctctgatgctgggcgaaacatctctcctctggggctcagttttctcatctgttagaaaaggacacagctgacctgttggcttctaatagttggacagaggctaggattctgagtctcattttactacaaatattcttttaatttcttaagtcactaaacagcatcagcaaggcagggtcgagacatgcgagcaagaatgagattggattctgactcaggtttcaacttgctgtcaattactgacaatgtaagttcattcatcttatagacttttgtagaacttttgtttctctccactataatttcgttactgttccatattacagtatgctaaagttaatggtaaaagttctcacagaattcctagtcttttcctcttcatatttaatctcctttccttcctcctgtccttactcattgtgaaattctcttttgtatgcatgacttggaaacatatttccttggtggtaaggtagtaggagacaatttattcacttttcacgtatgtcgtaattggcatattgctgataaagtttttcaaccatgggaacatggtcttgtaagaattatttcacatttttcccagtccaagcccataatgaaaattgattctgaattttttctgtatttttaattcttctgtttgcagttgtaggagaataaccctgcagcatctgagagaccaagctaattacaagaatgactagaaatcctttgcatttttaaaacaattttatacatatgtcactttgtctttctaaaaaataaaaataaaaaaaatacctaagagccgagtttgtgttaaaggctaatgattgtattgtacaattagtaagaattaaggacaaaggtctctttacctgaagtttcctgggtgcttttattcattcattcattcattcattcattcattcattcatttagtcaaattagttcatttctgatgcaatgactgactgattactccccagaccaatgctccttcctgttttaggttcacagatagcatttcctaccttctcttgtccttccttttgtccaaaattttgagttctagacaaccacagaattgcctagaaatgctggacagaattcatgcatctgattcctggtaagaccgtcgatgcactataaacttgcagaagctgacagcagactgttcttcacttcaactcatttatccctttcctttgggttctgtccaaatcacatcaccagatcacaagaacctaacatcagattgagacgtaaatagatgatatcacattggatttccaccattgagccacaccaccagccacctgcctgataactttcacagtcccagaagatattatacaagttactagggcaaaaagagatcaaagtctgaatcagctgtgaaccctatgaatggcaatacctacttatcaggcaatacaagcccacccgtgtgatagtggaataacagtaatatgggcaatcactggattgagtcctggccccactgcagagaatccatgccaagcactgtaaatccaggaagaaaaaaaaaaacctatcactgaagaagacataaaccctagaaaggaacttactactcttacttaactgagtgagcaaagcaacaagttatcttctaagtacttatgctggtgctcatacacaaaattatccatcattcttaattagagaattctctctagtgaatggttgtggattcaaagactcataaataccaagggtgctaagaatgagcgacaattaagaactcagccctaaacaagatttttatacctcatcttctaaggctcagaaacattgtggaagaaggtgtcaaaagaatgtaagagtgaaaagagtgagaagggctgccaatatcatctttgctatcatgaactcacaaaagctgcagttgttagtgccaggactgtgtgacattgtcactaccaacactcagccttgggtggggaggagggcataatgtcatactcttcatcattgagccattggttactaacagattctaggagaatcactctctcttgttatgtatccatccatgaatctacaaggctccattgggcagttccaaactggaggtcagaaaaatttcactgatgaaactcactgggacacaatcaaaaatatgaaagagctttgtagccatctttttttctgacaagggtgggagaggcataacaaggaaggtaaataattgattgcattatatacacatatgaaactgtcaaagaacgcaatttaaaaagtacatagtaagtggttttccatacaatttaatttattatcacacagttgttctttacagtatgtcttgattatctctatccctgactcccatgtcacccccacaaacaccctcaatatatctccctccaccttatcaccccttaatttctttcattttactattttatagataatccactgaattcaattagtgctgtctgttggaaagccgaaggagaccgatatgttggcttgatttgacacaggtcttctgcaggtgaccaagatgaagtgacttgaatgtgatagccatgctatgaaaaagagggcttcatgtattgtatcaaaagggagcgtttctcagctcctctctccagcctctgtctcatattctttctgctccgtcttcctctgtaacatagtaaatttgtacagaacggtcacaagtcacaaatttggtagactacatgatgaaatttgcaatgactttggagtacttaacatggatttgaatgtccatttggcatcgttctagaagataagtccaaagtaagtgtgctatcttaccatcttccttccttgtaggagtcggccacgtttcccactctagaccttagctcctctagttagctgcttcaaagcatcaagtggagtccgcataatcactttgtactaattcataagctcataaatccagacaaagtgaaagtcaaatctcaagtcctgggccacttatttgttttctgtgcatcggacttaggattatttgccctcttcctgttccactgcatcagttctgtcagtggggggggggggggttgggagtgtgtgtgtgtgtgtgtgtgtgtgtgtgtgtgtgtgtgtgtgtgttgcttacaaagctgtcataatgatgaaacagagtatcagtcacatggtaaccacatctaagtagagaatgtgcttctacaatgtgagcttcctctcagtgtgtccatgtcatcatagaggaggcttctttcccagtgcacatgaaggcttcagaactaagtttgaataggactatgtgatcagccctgaaaagcctgcagtactccttggtgctgtgcttgaaccctcctgtttctctgcgcggtctttgtagggagactatggatataaactatttgggtggtctcttttttttcatcaggaagacagaggtatactgttgattctagacatgtcaggttgaggaaatggaccttatgcctaattccttcctaattcatacagagtttcagctttaaaggacagattaatagcggtttgagatgatttcagctctgtgacctggccattgtgctgtgtgttagatttccatgctggtaagtgaaacaattttagggctctaaaaactcacttcaggctctaagcagcactccacctagccagaatgggggagatgcagctaaacagctgctcatgtgagcagggttaccaactccagtcgacagccaggccagcatgactcaccagtgtgaaactgccaagaggataatttgatctggggctgaatgaacaggactgcagtgtctgtccagaccaaagtgagggatcctcccttgtctgcatgtgaatccagaccacacctactgtcttgtaggctttgcttacccccacccctgtatctcattatgatgctgttcacaagttgaagtagagccagctatgagactcattgcataatattcacattagaaaccactctcttcattctatttctatcataggatttctaacttaacttgttgaaggtgtggatattgacatctttgagaagaagaaga

SEQ ID NO: 6 - DNA, 3949 bp, Chinese hamster
gatctgtgtagctgccacaacacttgatctcggagtgaggccctaactccattgatgggtgtcagctctcatcagtcgcactgttagcaacaggagatccagctgactgcctctcaagttatacagtgtgtgcaccagcttccaccacagcagctgctgctgtcagtttggaaataaagttcattcctaccttgcaggcactttggcatttgctttgggattatttgcacctcaggaagatccatcactagttttcattattctgaatgcaatggattatcagcctgtaaataatcaagtagacctcactggatttaaacattggaagctaagctatcaagcagatttatgaagttcacatgcttgtgcaatgtgagaagctgactttttggagctgcagtggcagccaaccaagcagcctgaggtttgttcttgaaagggagagtgtggactaaaggaagcctagaaagacacagaataaaatcaggagggcagatccagttaatactgaacaccacaagtttatttctcaccactctcatataccttaaccaaaaggtgaacatgagttccttcatacaaagcaaacactcttttcttgctgaatttttcaccaatttggtaaccataccttagattcaaattctagttacctgttctttagggacaggtgtcagcacatctcagaccaagtctgtttttatttagcataagacaccccatgccatgatgcaatatcctactgtagccacacctttgacctttaggttttatgatttcctaaggacagttatgaactctctgcccttgagccaagatggagtccagccgtctttatgggaactagcagtgcaatgtgattctctcatccattgcattcgtcaaaaggcaattgtgagtaaagggaggatgtagtggttcatctatttgcctgactgatatcctaacagctcccctagtttttaatttttttttagttcttgtgaagatgtcatggctggtctggagctcctgggtatactgtagcctattttactgtctaagcctctggggtagctgggattgctggatcatggtgacaggtaactcactacccaattttaaagtgaatttgtaatgaaaggatgatgattgttacctacttgttagggctaggaattgatttcttcccaacattttagagattttccctgtgtattaatggcatttatcttgcatctacaattgatgctgttcaaagctgcccaggctggcctctaactcacagagatgcaaatgcctctgcctcccgagtgctgggattaaaggcgtgcaccactaatgcctggctctttttaaaatcttttaggttattgcttcctaagctctagtgactatgggtagatatcaaagacaatacagttttcattggttctgttttggtgtgtagtttttgttggctactttcttctttacacagatttcatgtagtgcacactcatcttgagctctctacatagcacaagaggaccttgcaggcttgattatccagccgctaattcctaagtgctgagtgacaagtgtgtgacactgtgcctctcattttgttggttattttagaaagagtcttactaagttgcccagactaggctcaaactctgaatatctcccagctttagcctccatagtcttgcatttacaggcagtttaatcttgagctaacagtccctgctgataccaagtttttattctaggtgtccaagaggaactgtagcagtgaactccagtctagccaaagacacttgaccattgcactctggatcttgtctttagatatgtattttgggggatttctttttaatcaacaggaaatcaaataaacttaaaaaagaatttacgcaggcagcactggttcaagtatttaatctcaacaccctgtagatataggcaaaagtatctctgagcagaaagatagccagggttacaaagagaaaaactgtctcaaaaattatatatatgtgagtgagtgtgtgcgtgttagttattttaaattatatgtataaatgtacatgcatatgcaagagcccatggagatcaggagaaattgtgttctctaagagctgtagttactggtgggtgaaagccaccagggttgggagagagaaatagaactgtagtactatgatagaacaagaagtgctcttaacctgagttatggttctagctcaatagatacactattcacagttattttaaagatactgttgttgttgtcttttactgtgcatttgggtgataaaacatgatccaacacactcaacaaatccacatggagtttattggaaaagggaataaagggaggggtaggtgttaaccaatagggagcagaaatggaaagagagaaaacagatgggaggcacttgcttataaagggaaaggaaacagttaagaatgaggctcagtagttggggcctttgaaaccatagtcactgaactgcctttggccaagatttacatggtctctgtatgcagaatcctaattcagtcaattaacacatgcaccacacagccatgcaaactttgacagtctttgagatgtcagcaaggaacaatcacctgtgaaaaacagatcccagggcaagggcaggtcacctggaaaagagaagagaagatggatcccagagcagggagggaatccaagtgttagagaggccactaggccaggaaaggatctctaaggaagcaacaggcccaggagagtgctgatgtggagtgacatgtggagatcaagagaaaacaccagggtgggaggagagaaattggcagctggatcagggccaggtcgcacagaacctagggagagggagaatccaggttatcaacaattattactaggcagtactacattttctgtgtcctattatttctgtagttacttacaaaatatttgagttataaaaaggaataaagagccgggcagtggtggcacatggcattaacaccagcacttgggagacacaggcagttgcatctatgtgagtttgaggccagcctggtctacagagggagtcccaggaccaaaagccacagagtaactttgtcatacaaactgatccagtaggcttcatctcagatacgcagtgatggttcaacatacaaaaatcagtaactgtaatccaccataaaaataaactttaaaaaacacttttttattatccctttacatgcttacaaagtcattgataagccaggtattgggggtgcatgcctttaatcccagtacttgggaggcagaggcaggtggatcactgtgagttcaaggccagcctgatctccagagcgagtgccaggataggcttcaaagctgcacggagaaaccctgtcttgaaaaaccaataaataaataaataaataaatagtcattgacaagaaacaaacatcataaaagtcttggagatattatggatacaatttacatacacacacataatgaaggacatttacagcaaacctatagacaacatcaaatacaatggagagaaaaaacaaaggaattcctataaaatctgtaacttgacaagtttgtgaagtctatatctactcaatacagtacttgaagttctagatagacccattaaacagctaaaggacaacaaggaaaggaagaagtagaagtgttgttacttgttgatgatatagtggtaccacctaagtgacactaaaaattcatcaatggaagtacaggtgattaaaactttcagcaaagtgacgggatacaagagtaactaaaacaaccattagccctcctatgtaaaaatggcaaacagcttgagaatgaaataaaagaagcagcagcaatcacaatagcttcaaataatataaaatacattctagtaactctaacttgtttaattaaaaaaactttaagtgtttgaagaaagaaattgaagaagatatgaggcgatggaaa

SEQ ID NO: 7 - DNA, 1128 bp, Chinese hamster
gatcaggagttcaaggccacactgaggtacacgaaattcaaccagtctgatagatataagagctgggtgcgtgtggctcgcacctcaggtggagacaggagtataaggctggaggaggcagtatttaggcttattcatatagaggatttgtaaagacaggacctccccagcacttccatctgaacatttggtacaggtaagaagtccctatagagttggctcctttaattctcttatgtctcaacatttacccaattatctgacatctcactcagcgtttttactatttaaaccaatttgaagaaatgctacagagcaccttttaacctctacaaacacacataaacacagagagagagagagagagagagagagagagagagagagagacagagacagagacagagacagagacagagacagagaaacaaatgtaataacgaaagaagtcatgtcatgagaaccctgaggctgcggtccacacccatctgtggccaggacacagaggcctagaggagccctgtgacacaagcactctctacaactggcccttgtcccgtgcagggggcagaaaggacagattttgttgtgcagaagctttatcatcagcagcatacactgggcctctctgtccttcactgtcacatgctcctagggagttcagtcgggaggtcatgtatgtgcactatggacctgtcccacagacactctgtcctaatgcgttctgctggggtattttggcaatgctgcaattgagcagtgatgtttcaaggtgcactagttgttccccccatattctccaacacaatcaatgccacattgtaaatcaaaacattcaggctcccctgtgaattgtaaggattttattattggaatcctggttttagatacctggagggtagggtagggcttgcttcatctattcaggtgtgtaggcaagtggctcccttgagtcttattgcccagatggattcatcaacagaatttgttagcatctattttctgctgcaaagagaacccggtgaggtatctgaggtgtcagaggtgaaggacatctcactgagcatacatgggacacctcatgggagggactgaaacctgtctgccagagcacctgggtctgaccat

SEQ ID NO: 8 - DNA, 1352 bp, Chinese hamster
gatctctcagcttcctgctttttaaaagtattttattttatttttatacccattgatgttttttgtcgtgggtgtcggataccctgaaactggaggttttcattttatatttatgttaatcaatgttttgccatgggtgttgcgtcccctgaaactggagctacagacaggtgtgagctgccatgtggggctgggaactgaacttgagtcctctggaagaggagtcagtgctcttaactagtgagccatctctctaggccctcagcttcctgctttggctaccagctgacatgcctctcccaccattatgaatgccccctcaggaacctctggaactgaaaaccaaaataaactttttaaagttgctttagttcatggcattttatcacaacaatagacaagaaactaatacagtaatacatggctttttaaatgatttgacagattcatgtaagtatatagtgaatttgggtcatttttcaccctttaataccattgtcatcctccttcctaaccagctgggaccctcttcctcagcaggccctcttctactttcattttttttttttttttttgtgtgtgtgtgtgtgtgtgtgtgtatgtgtgctcgcgcgtgtgctgtgtccttatgtttatttatataaaaaatagcgcattgactctaacttttactacaccttactggttatatatgtatgtgtatgccatggtacatgtgcagagaacaaaggacaactttccgggagtcatttctatccttccactatgcatgtggtttctgggatagaactcaggtcattagccttggcagcaagcctcttaaccctctgaaccatctccctggcctggcattttaaaataatctttgatgcttctatcagtatcttggccactgataatctataattatttctctaagactatttgttttccacaaacaaaatgctataagctgggagatttataaagaagagatacatttggctcacagctctggaaactgggaagtccaaaagcatgacaccagcagctgtcaaatgcctttctgcagtatcataagaaatcagaggacagcacatgacaagaatgttacaaaaggacaggacaagtgttccaggcttggtctatggttttcatcatttaaggccgccaattccatcacaagtgttctcttccctatgatttcatgtaattctaaagacattctaaaaccccacacccaaatactattagcacaagacattggagattttagtttcaatcttagctttaggggagagacactcagttcataacagtatccccaagatttccagtatccagtgctgtctcaatgcaatactactcagaag

SEQ ID NO: 9 - DNA, 1246 bp, Chinese hamster
gatctttccattttctggtatcttctttaatttctttcttttaagactcaaagttcttgctagacaggtctttcacttgtttggttatcattaccccaagatattttatgttgtttggctattgtaaaggatgatgtttctctgatttatttctcagcccatttatctcctgtgtataatagggctagtgattttttgagttaatcttgtatccttccacttagctgaaggtgtttatcagctgtagtagttccctggtagagttttttgggttacttatgtaactatcatatcatctgcaaacagtaaaaatttgacttcttcctttccaatttgtatccccttgttctcctttttgttgtcatattgccccagatagaacttcaagtacaagcagaagtcattctcttctgcttcatctgtgttgggatgttcaggtcttgctggcgtagagtccctagattctagtggtgtcatattgttttttctgttattgaatgcgtttttatattgttgtcttcccatctcttcttccagtgggttcaggtgccgtctcttcctctcctggtgtgtatgggtccaaggttctctttggtggatgcaagagggtctgatactctgatgggtcttatggtgggttcaggcgggtctggggcactccctctctaggtgggggtgggaactggactagcacagtgatgtcatcagacttgaggttgcttggtcctcagggggcaagttgatttgcctgcagtccccaggacaggagttcccagagtggacaggcagaagtcgggctcaaggcaggggccaagctctacatgtgatttttaaaatgagagttcagattcatgtaggcagatgataagctcagggagagaaatgacctatttctaaaaactgatgacgtgaagattgagagaaagggtggatttttgaaaaagaatcggtagggagctaaaaaggaaaagagaaattaaggatgactctcaggttttggacttgaatgttggatggatgtttgtcccatttgtagaaaggagaacacaggtgatttagaagtctgaggtgaggatgtcacctcatgacttaaagaatctgaggttttagaatcaaatctcagggaacatcattagcagagggaccctgttgggtcttgccagatgctgagcttcagctgtctcctgttttcccacatttcctgtttttcctaacttgtatagactctgggaaaagaaggtaccag

SEQ ID NO: 10 - protein, 447 aa, Homo sapiens
FTVTVPKDLYVVEYGSNMTIECKFPVEKQLDLAALIVYWEMEDKNIIQFVHGEEDLKVQHSSYRQRARLLKDQLSLGNAALQITDVKLQDAGVYRCMISYGGADYKRITVKVNAPYNKINQRILVVDPVTSEHELTCQAEGYPKAEVIWTSSDHQVLSGKTTTTNSKREEKLFNVTSTLRINTTTNEIFYCTFRRLDPEENHTAELVIPELPLAHPPNERTPRDCGCKPCICTVPEVSSVFIFPPKPKDVLTITLTPKVTCVVVDISKDDPEVQFSWFVDDVEVHTAQTQPREEQFNSTFRSVSELPIMHQDWLNGKEFKCRVNSAAFPAPIEKTISKTKGRPKAPQVYTIPPPKEQMAKDKVSLTCMITDFFPEDITVEWQWNGQPAENYKNTQPIMDTDGSYFVYSKLNVQKSNWEAGNTFTCSVLHEGLHNHHTEKSLSHSPGK

SEQ ID NO: 11 - protein, 451 aa, Artificial Sequence
EVQLVESGGGLVQPGRSLRLSCAASGFTFDDYAMHWVRQAPGKGLEWVSAITWNSGHIDYADSVEGRFTISRDNAKNSLYLQMNSLRAEDTAVYYCAKVSYLSTASSLDYWGQGTLVTVSSASTKGPSVFPLAPSSKSTSGGTAALGCLVKDYFPEPVTVSWNSGALTSGVHTFPAVLQSSGLYSLSSVVTVPSSSLGTQTYICNVNHKPSNTKVDKKVEPKSCDKTHTCPPCPAPELLGGPSVFLFPPKPKDTLMISRTPEVTCVVVDVSHEDPEVKFNWYVDGVEVHNAKTKPREEQYNSTYRVVSVLTVLHQDWLNGKEYKCKVSNKALPAPIEKTISKAKGQPREPQVYTLPPSRDELTKNQVSLTCLVKGFYPSDIAVEWESNGQPENNYKTTPPVLDSDGSFFLYSKLTVDKSRWQQGNVFSCSVMHEALHNHYTQKSLSLSPGK

SEQ ID NO: 12 - protein, 214 aa, Artificial Sequence
DIQMTQSPSSLSASVGDRVTITCRASQGIRNYLAWYQQKPGKAPKLLIYAASTLQSGVPSRFSGSGSGTDFTLTISSLQPEDVATYYCQRYNRAPYTFGQGTKVEIKRTVAAPSVFIFPPSDEQLKSGTASVVCLLNNFYPREAKVQWKVDNALQSGNSQESVTEQDSKDSTYSLSSTLTLSKADYEKHKVYACEVTHQGLSSPVTKSFNRGEC

SEQ ID NO: 13 - DNA, 943 bp, Homo sapiens
gtaagtgccgtgtgtggttcccgcgggcctggcctctttacgggttatggcccttgcgtgccttgaattacttccacgcccctggctgcagtacgtgattcttgatcccgagcttcgggttggaagtgggtgggagagttcgaggccttgcgcttaaggagccccttcgcctcgtgcttgagttgaggcctggcttgggcgctggggccgccgcgtgcgaatctggtggcaccttcgcgcctgtctcgctgctttcgataagtctctagccatttaaaatttttgatgacctgctgcgacgctttttttctggcaagatagtcttgtaaatgcgggccaagatctgcacactggtatttcggtttttggggccgcgggcggcgacggggcccgtgcgtcccagcgcacatgttcggcgaggcggggcctgcgagcgcggccaccgagaatcggacgggggtagtctcaagctggccggcctgctctggtgcctggcctcgcgccgccgtgtatcgccccgccctgggcggcaaggctggcccggtcggcaccagttgcgtgagcggaaagatggccgcttcccggccctgctgcagggagctcaaaatggaggacgcggcgctcgggagagcgggcgggtgagtcacccacacaaaggaaaagggcctttccgtcctcagccgtcgcttcatgtgactccacggagtaccgggcgccgtccaggcacctcgattagttctcgagcttttggagtacgtcgtctttaggttggggggaggggttttatgcgatggagtttccccacactgagtgggtggagactgaagttaggccagcttggcacttgatgtaattctccttggaatttgccctttttgagtttggatcttggttcattctcaagcctcagacagtggttcaaagtttttttcttccatttcag

SEQ ID NO: 14 - protein, 447 aa, Artificial Sequence
QVQLVQSGVEVKKPGASVKVSCKASGYTFTNYYMYWVRQAPGQGLEWMGGINPSNGGTNFNEKFKNRVTLTTDSSTTTAYMELKSLQFDDTAVYYCARRDYRFDMGFDYWGQGTTVTVSSASTKGPSVFPLAPCSRSTSESTAALGCLVKDYFPEPVTVSWNSGALTSGVHTFPAVLQSSGLYSLSSVVTVPSSSLGTKTYTCNVDHKPSNTKVDKRVESKYGPPCPPCPAPEFLGGPSVFLFPPKPKDTLMISRTPEVTCVVVDVSQEDPEVQFNWYVDGVEVHNAKTKPREEQFNSTYRVVSVLTVLHQDWLNGKEYKCKVSNKGLPSSIEKTISKAKGQPREPQVYTLPPSQEEMTKNQVSLTCLVKGFYPSDIAVEWESNGQPENNYKTTPPVLDSDGSFFLYSRLTVDKSRWQEGNVFSCSVMHEALHNHYTQKSLSLSLGK

SEQ ID NO: 15 - protein, 218 aa, Artificial Sequence
EIVLTQSPATLSLSPGERATLSCRASKGVSTSGYSYLHWYQQKPGQAPRLLIYLASYLESGVPARFSGSGSGTDFTLTISSLEPEDFAVYYCQHSRDLPLTFGGGTKVEIKRTVAAPSVFIFPPSDEQLKSGTASVVCLLNNFYPREAKVQWKVDNALQSGNSQESVTEQDSKDSTYSLSSTLTLSKADYEKHKVYACEVTHQGLSSPVTKSFNRGEC

SEQ ID NO: 16 - DNA, 680 bp, human cytomegalovirus
gttgacattgattattgactagttattaatagtaatcaattacggggtcattagttcatagcccatatatggagttccgcgttacataacttacggtaaatggcccgcctggctgaccgcccaacgacccccgcccattgacgtcaataatgacgtatgttcccatagtaacgccaatagggactttccattgacgtcaatgggtggagtatttacggtaaactgcccacttggcagtacatcaagtgtatcatatgccaagtacgccccctattgacgtcaatgacggtaaatggcccgcctggcattatgcccagtacatgaccttatgggactttcctacttggcagtacatctacgtattagtcatcgctattaccatggtgatgcggttttggcagtacatcaatgggcgtggatagcggtttgactcacggggatttccaagtctccaccccattgacgtcaatgggagtttgttttggcaccaaaatcaacgggactttccaaaatgtcgtaacaactccgccccattgacgcaaatgggcggtaggcgtgtacggtgggaggtctatataagcagagctcgtttagtgaaccgtcagatcgcctggagacgccatccacgctgttttgacctccatagaagacaccgggaccgatccagcctccggactcta

SEQ ID NO: 17 - DNA, 3619 bp, Chinese hamster
ttaattaccgacaatggctggtacagcaagtagcacggaaaaaaagtgaaacagttgcactgttcatggttggcaataattcttcaggaaaatatttactatcaatcagttatgagaaaagggactctgtgctcgtaaaacagcacgttgcttctcataccaggaccattttgcttcagcataatctgaatttaaacagcttgtttcctgcggatataattttggaaataaataaaacaagtcttctatcaaaatccggagtgagtgggaaggaacatcacatctttctatctcagtcagtttcaaacagattattagtcccaagtaaaaaacagtaataacaaacaacaaaaatacagaatgtacacaaggccactgatgggcttattccaaagaaagacagacctttcccactgtaggccaggtatcaaggtagaagtgcccgaacaattcaattttaactgcacatgtttatggaaggggtgtgaggtgtaagggtaaattatggaaaagcctcaaaccaaaattttctgtagtatttcaataaagtcaataacaagataacataaaaattaatgttctcagtttttttcataattaaaaaacatgaaggttgacaattaggtacaatgtgattatagattttaaagactaagctgacagtcaataaccgctgtccatttaaagctacaataaatatagagctcatcatgttccccaaacaaatcccataaagcaccagggctgtgagcagcagatgagatgctctaaaaagcaaactagctggcatggtggtgcatccagcacttgggaggcggaggcaggtggatttctgtgagttcaaggacagcctggttgatatggccaaagctacatcggacagacagacagacaaaacaaaacaaaaaagcaaactatattcaagatatttcatggcttcaaatactacttggacccctccccatttttatttttaaatgtttctttcttgaactctttctttcaggagactgctgtcagcctaaggtagcttatgaagcagctgtgcttccttacaggaactgaatagttacagggcaaccagcagaggaaaactacacacaaaatactacaggtttcatctctgcttttgagaaggaccaatgtcttctgtaaaatgcaaacaagtaataattaaaaggtctaagactacaattagtattgatacccaaaccaaaattactctgactgaaattcagttgctttgaaccataagggggaaaaaaaggctggcttcactgtatttcagtggcgttacatggagacagctggacatgtaggccacaatggagaccagtttgaatcagtatcagacgccagtttctgaaggaaagtcctcacagccacgtcagtgtagcagacaaaactactgttaagaactaaaggtgaagaacaagaactagagaaatgcttacagaactacaaaaatatctttgagtcatttcttttaaaggtcaagcagtaaatgaggccaggagagacagtatgaaatcatgagacagatataacatgtttagcaataagaaaggaaaactctcattgttgccatgctagaggaggccactgcaataaacatttttttcagttacgtatttttatttgatgatttggctcaaatctgaagcaatgaactagaagacaggatgtgggccaataaaaggaaccaggaagctggttgtgttccaaatggaaattacagaaatcattattcaattagagtggttaaggggacaatgaaagaaaataggtgtcagaataatgttaaaacaagcaagaatgggacgagaaggtcaccatctgggagcaagtgaaacagactgatgagcagcaatgagcaaacttatttcctcacccaagagcatggaaggaattataccaccgtgccagacgccacaagatttctaaccgtgcaccactgaagtagagggtagaaaaaagaaaaaagaacagcaaaaacaaatccaccccacactatacacacagcaacaaggctaaggagtgtagaaacactggcttaccacgtacaggaaaacaaaaggaacagatgctcagttggccagctctcaatgaaactcattaaaattgtcgccctgtccttggattggtggtcatgcgaaatttgtgccttgtttagccagaagtaacttgtgatgaaggagagaacagcatgtccaaacaagaattgaaacacttgttgatctatactcaatgctagatataaaacaggatcaagtagcacttacaaactgttactaagtaattgaaaattaaatgtaacttacactactcctcttttttttttgtagcaaattaagatgtgaacttaaggcacaatttgatgaacctaccatttgcagctacaatataaaataaattcttacatttctcatatggctaagtccaatggccacaagctgtatgtttgcagtaataaagcaaggtcaggaactgccatgtattttgggaaatataataaaaattattgttgctcctatgtcctgattgatcatgtccctccctaaccacctaatgtgtaagaacagagtctccatgaacagaattagagcactatgcaataagtaaatgaatgaacagattaataagagatcccagagggcttagctcatcccttccatcctgagattatattatagcaaggattccatctatgaagaagagtcaacttccaactagacattgaatctactgtcaccatgatcttcccatatctagaactataaaaataagtcactgtttataagctaccttgtttatttttggttgtaataacacaaaagaaattagctcttcttgagatttataacaaagatggagttgacatgacatcaagtcctatctctaataatgacagtaaataggggcctatataggacacaagagatgaagcagaaagttggaaaagttgtaaaacagtcaccccccaaaatggtaataaaggttatttttgcctaaaaataaagacaaactctagaaatacaactcatactgaacgttatcctcaagacagtaaagttaacaaaaaagttatccccagtcaatctagaaaattgaaagaaaaaaattaagatttctaattaaatttttgtgtatgggtgttttgtctatatgtatgtctgtagaggccagaagaagacactgggtcctctggaacgggagctgcagatggttgagagccgtcatacggtgctgacaggtaacccgggtcctatacaggagcagcccttaaccaatgagctcttaaccaatgaacccctctccagccctgaagatttctaatttttaatatttttgtatctagaaatataacacacatttatacataaaagactaggctcatatgtcagctaaatacatgtttccactcaaaatcaccaagtaagacatttctcaagaaagaagggcacaacctaagctgggacctctgcagcagtctcacgcatgtggctcacactgtcaccagcagggtatttctggcgtgctacacctgcacttaaaggaggccaggcatggcggtgctggcctttaatcccagcactcacggggcagaggcaggcagatc

SEQ ID NO: 18 - DNA, 1114 bp, Chinese hamster
tccacactcatgttgacattaaagccatcgacaatctcagtaagtactagtaaacaagtaacaaataagactgatccatcacacaacattaccctggctgtgtctttggagtaaaaatcatgtagatcaaggtatggtatgcttgaacaccaaaaagtaaccacagagtagaagagtagagtccagtgagtgccttatgcgtgagcccacttccctttttgcgtttgtttttacttaatgtctggcagaattcaggcatgtaggtcagaggccaccttgcaggagtccgttctctctttccaccaactggatcccagggacaggacacaggtcttgggcttggcagcgggtgcccttacctactgagccatttcaccactgacttggttttactgaaagctaactctgaagactggaattcgatacttttttagggtgatgagtcactcactgtacagcctcagcactattgctgaagtacattaccctcacaaaccaggcagccggagactcactgcttacatgtaatcgaggccatgctatgttaggtaacatgttggagacttaccaaaaactgtgttttaaagttacttgcaacctttctgtaaccacgcaaactgctgtgtgattctttaacctatgtctccacaatcacaacagacatctgttccgggtaattgcacatttctaattaaagctttcaaagtgggccaggttctctggagctgaaatgttcgttgaagggggcaaagttattttctctaacatcatgagggaactgggtcagggtgtggggactgcaccctgctgaggggatggtataggaatgacccacctttggcctgtgttccttttgttttgctttgtgcatgtgtttgcatttctgtttgcatgcaagtgagctcatttgctgtggaagcccaaagctgatgtcactctctatcttattcactgaaccagagtcgctccacgaacccagagctctcagctaacactagcctagctagccagctgcccttgggatcctttctcagccttccaagtgctgaaattgcaggtacactactaagcccgtaggcctttgtgtgggttctgcagatccaaacttcagatc

SEQ ID NO: 19 - DNA, 4068 bp, Chinese hamster
tcttcttcttctcaaagatgtcaatatccacaccttcaacaagttaagttagaaatcctatgatagaaatagaatgaagagagtggtttctaatgtgaatattatgcaatgagtctcatagctggctctacttcaacttgtgaacagcatcataatgagatacaggggtgggggtaagcaaagcctacaagacagtaggtgtggtctggattcacatgcagacaagggaggatccctcactttggtctggacagacactgcagtcctgttcattcagccccagatcaaattatcctcttggcagtttcacactggtgagtcatgctggcctggctgtcgactggagttggtaaccctgctcacatgagcagctgtttagctgcatctcccccattctggctaggtggagtgctgcttagagcctgaagtgagtttttagagccctaaaattgtttcacttaccagcatggaaatctaacacacagcacaatggccaggtcacagagctgaaatcatctcaaaccgctattaatctgtcctttaaagctgaaactctgtatgaattaggaaggaattaggcataaggtccatttcctcaacctgacatgtctagaatcaacagtatacctctgtcttcctgatgaaaaaaaagagaccacccaaatagtttatatccatagtctccctacaaagaccgcgcagagaaacaggagggttcaagcacagcaccaaggagtactgcaggcttttcagggctgatcacatagtcctattcaaacttagttctgaagccttcatgtgcactgggaaagaagcctcctctatgatgacatggacacactgagaggaagctcacattgtagaagcacattctctacttagatgtggttaccatgtgactgatactctgtttcatcattatgacagctttgtaagcaacacacacacacacacacacacacacacacacacacacacacacactcccaaccccccccccccccactgacagaactgatgcagtggaacaggaagagggcaaataatcctaagtccgatgcacagaaaacaaataagtggcccaggacttgagatttgactttcactttgtctggatttatgagcttatgaattagtacaaagtgattatgcggactccacttgatgctttgaagcagctaactagaggagctaaggtctagagtgggaaacgtggccgactcctacaaggaaggaagatggtaagatagcacacttactttggacttatcttctagaacgatgccaaatggacattcaaatccatgttaagtactccaaagtcattgcaaatttcatcatgtagtctaccaaatttgtgacttgtgaccgttctgtacaaatttactatgttacagaggaagacggagcagaaagaatatgagacagaggctggagagaggagctgagaaacgctcccttttgatacaatacatgaagccctctttttcatagcatggctatcacattcaagtcacttcatcttggtcacctgcagaagacctgtgtcaaatcaagccaacatatcggtctccttcggctttccaacagacagcactaattgaattcagtggattatctataaaatagtaaaatgaaagaaattaaggggtgataaggtggagggagatatattgagggtgtttgtgggggtgacatgggagtcagggatagagataatcaagacatactgtaaagaacaactgtgtgataataaattaaattgtatggaaaaccacttactatgtactttttaaattgcgttctttgacagtttcatatgtgtatataatgcaatcaattatttaccttccttgttatgcctctcccacccttgtcagaaaaaaagatggctacaaagctctttcatatttttgattgtgtcccagtgagtttcatcagtgaaatttttctgacctccagtttggaactgcccaatggagccttgtagattcatggatggatacataacaagagagagtgattctcctagaatctgttagtaaccaatggctcaatgatgaagagtatgacattatgccctcctccccacccaaggctgagtgttggtagtgacaatgtcacacagtcctggcactaacaactgcagcttttgtgagttcatgatagcaaagatgatattggcagcccttctcactcttttcactcttacattcttttgacaccttcttccacaatgtttctgagccttagaagatgaggtataaaaatcttgtttagggctgagttcttaattgtcgctcattcttagcacccttggtatttatgagtctttgaatccacaaccattcactagagagaattctctaattaagaatgatggataattttgtgtatgagcaccagcataagtacttagaagataacttgttgctttgctcactcagttaagtaagagtagtaagttcctttctagggtttatgtcttcttcagtgataggtttttttttttcttcctggatttacagtgcttggcatggattctctgcagtggggccaggactcaatccagtgattgcccatattactgttattccactatcacacgggtgggcttgtattgcctgataagtaggtattgccattcatagggttcacagctgattcagactttgatctctttttgccctagtaacttgtataatatcttctgggactgtgaaagttatcaggcaggtggctggtggtgtggctcaatggtggaaatccaatgtgatatcatctatttacgtctcaatctgatgttaggttcttgtgatctggtgatgtgatttggacagaacccaaaggaaagggataaatgagttgaagtgaagaacagtctgctgtcagcttctgcaagtttatagtgcatcgacggtcttaccaggaatcagatgcatgaattctgtccagcatttctaggcaattctgtggttgtctagaactcaaaattttggacaaaaggaaggacaagagaaggtaggaaatgctatctgtgaacctaaaacaggaaggagcattggtctggggagtaatcagtcagtcattgcatcagaaatgaactaatttgactaaatgaatgaatgaatgaatgaatgaatgaatgaatgaataaaagcacccaggaaacttcaggtaaagagacctttgtccttaattcttactaattgtacaatacaatcattagcctttaacacaaactcggctcttaggtattttttttatttttattttttagaaagacaaagtgacatatgtataaaattgttttaaaaatgcaaaggatttctagtcattcttgtaattagcttggtctctcagatgctgcagggttattctcctacaactgcaaacagaagaattaaaaatacagaaaaaattcagaatcaattttcattatgggcttggactgggaaaaatgtgaaataattcttacaagaccatgttcccatggttgaaaaactttatcagcaatatgccaattacgacatacgtgaaaagtgaataaattgtctcctactaccttaccaccaaggaaatatgtttccaagtcatgcatacaaaagagaatttcacaatgagtaaggacaggaggaaggaaaggagattaaatatgaagaggaaaagactaggaattctgtgagaacttttaccattaactttagcatactgtaatatggaacagtaacgaaattatagtggagagaaacaaaagttctacaaaagtctataagatgaatgaacttacattgtcagtaattgacagcaagttgaaacctgagtcagaatccaatctcattcttgctcgcatgtctcgaccctgccttgctgatgctgtttagtgacttaagaaattaaaagaatatttgtagtaaaatgagactcagaatcctagcctctgtccaactattagaagccaacaggtcagctgtgtccttttctaacagatgagaaaactgagccccagaggagagatgtttcgcccagcatcagagcctttcaactcagagccagacctagaagatc

SEQ ID NO: 20 - DNA, 3949 bp, Chinese hamster
tttccatcgcctcatatcttcttcaatttctttcttcaaacacttaaagtttttttaattaaacaagttagagttactagaatgtattttatattatttgaagctattgtgattgctgctgcttcttttatttcattctcaagctgtttgccatttttacataggagggctaatggttgttttagttactcttgtatcccgtcactttgctgaaagttttaatcacctgtacttccattgatgaatttttagtgtcacttaggtggtaccactatatcatcaacaagtaacaacacttctacttcttcctttccttgttgtcctttagctgtttaatgggtctatctagaacttcaagtactgtattgagtagatatagacttcacaaacttgtcaagttacagattttataggaattcctttgttttttctctccattgtatttgatgttgtctataggtttgctgtaaatgtccttcattatgtgtgtgtatgtaaattgtatccataatatctccaagacttttatgatgtttgtttcttgtcaatgactatttatttatttatttatttattggtttttcaagacagggtttctccgtgcagctttgaagcctatcctggcactcgctctggagatcaggctggccttgaactcacagtgatccacctgcctctgcctcccaagtactgggattaaaggcatgcacccccaatacctggcttatcaatgactttgtaagcatgtaaagggataataaaaaagtgttttttaaagtttatttttatggtggattacagttactgatttttgtatgttgaaccatcactgcgtatctgagatgaagcctactggatcagtttgtatgacaaagttactctgtggcttttggtcctgggactccctctgtagaccaggctggcctcaaactcacatagatgcaactgcctgtgtctcccaagtgctggtgttaatgccatgtgccaccactgcccggctctttattcctttttataactcaaatattttgtaagtaactacagaaataataggacacagaaaatgtagtactgcctagtaataattgttgataacctggattctccctctccctaggttctgtgcgacctggccctgatccagctgccaatttctctcctcccaccctggtgttttctcttgatctccacatgtcactccacatcagcactctcctgggcctgttgcttccttagagatcctttcctggcctagtggcctctctaacacttggattccctccctgctctgggatccatcttctcttctcttttccaggtgacctgcccttgccctgggatctgtttttcacaggtgattgttccttgctgacatctcaaagactgtcaaagtttgcatggctgtgtggtgcatgtgttaattgactgaattaggattctgcatacagagaccatgtaaatcttggccaaaggcagttcagtgactatggtttcaaaggccccaactactgagcctcattcttaactgtttcctttccctttataagcaagtgcctcccatctgttttctctctttccatttctgctccctattggttaacacctacccctccctttattcccttttccaataaactccatgtggatttgttgagtgtgttggatcatgttttatcacccaaatgcacagtaaaagacaacaacaacagtatctttaaaataactgtgaatagtgtatctattgagctagaaccataactcaggttaagagcacttcttgttctatcatagtactacagttctatttctctctcccaaccctggtggctttcacccaccagtaactacagctcttagagaacacaatttctcctgatctccatgggctcttgcatatgcatgtacatttatacatataatttaaaataactaacacgcacacactcactcacatatatataatttttgagacagtttttctctttgtaaccctggctatctttctgctcagagatacttttgcctatatctacagggtgttgagattaaatacttgaaccagtgctgcctgcgtaaattcttttttaagtttatttgatttcctgttgattaaaaagaaatcccccaaaatacatatctaaagacaagatccagagtgcaatggtcaagtgtctttggctagactggagttcactgctacagttcctcttggacacctagaataaaaacttggtatcagcagggactgttagctcaagattaaactgcctgtaaatgcaagactatggaggctaaagctgggagatattcagagtttgagcctagtctgggcaacttagtaagactctttctaaaataaccaacaaaatgagaggcacagtgtcacacacttgtcactcagcacttaggaattagcggctggataatcaagcctgcaaggtcctcttgtgctatgtagagagctcaagatgagtgtgcactacatgaaatctgtgtaaagaagaaagtagccaacaaaaactacacaccaaaacagaaccaatgaaaactgtattgtctttgatatctacccatagtcactagagcttaggaagcaataacctaaaagattttaaaaagagccaggcattagtggtgcacgcctttaatcccagcactcgggaggcagaggcatttgcatctctgtgagttagaggccagcctgggcagctttgaacagcatcaattgtagatgcaagataaatgccattaatacacagggaaaatctctaaaatgttgggaagaaatcaattcctagccctaacaagtaggtaacaatcatcatcctttcattacaaattcactttaaaattgggtagtgagttacctgtcaccatgatccagcaatcccagctaccccagaggcttagacagtaaaataggctacagtatacccaggagctccagaccagccatgacatcttcacaagaactaaaaaaaaattaaaaactaggggagctgttaggatatcagtcaggcaaatagatgaaccactacatcctccctttactcacaattgccttttgacgaatgcaatggatgagagaatcacattgcactgctagttcccataaagacggctggactccatcttggctcaagggcagagagttcataactgtccttaggaaatcataaaacctaaaggtcaaaggtgtggctacagtaggatattgcatcatggcatggggtgtcttatgctaaataaaaacagacttggtctgagatgtgctgacacctgtccctaaagaacaggtaactagaatttgaatctaaggtatggttaccaaattggtgaaaaattcagcaagaaaagagtgtttgctttgtatgaaggaactcatgttcaccttttggttaaggtatatgagagtggtgagaaataaacttgtggtgttcagtattaactggatctgccctcctgattttattctgtgtctttctaggcttcctttagtccacactctccctttcaagaacaaacctcaggctgcttggttggctgccactgcagctccaaaaagtcagcttctcacattgcacaagcatgtgaacttcataaatctgcttgatagcttagcttccaatgtttaaatccagtgaggtctacttgattatttacaggctgataatccattgcattcagaataatgaaaactagtgatggatcttcctgaggtgcaaataatcccaaagcaaatgccaaagtgcctgcaaggtaggaatgaactttatttccaaactgacagcagcagctgctgtggtggaagctggtgcacacactgtataacttgagaggcagtcagctggatctcctgttgctaacagtgcgactgatgagagctgacacccatcaatggagttagggcctcactccgagatcaagtgttgtggcagctacacagatc

SEQ ID NO: 21 - DNA, 1128 bp, Chinese hamster
atggtcagacccaggtgctctggcagacaggtttcagtccctcccatgaggtgtcccatgtatgctcagtgagatgtccttcacctctgacacctcagatacctcaccgggttctctttgcagcagaaaatagatgctaacaaattctgttgatgaatccatctgggcaataagactcaagggagccacttgcctacacacctgaatagatgaagcaagccctaccctaccctccaggtatctaaaaccaggattccaataataaaatccttacaattcacaggggagcctgaatgttttgatttacaatgtggcattgattgtgttggagaatatggggggaacaactagtgcaccttgaaacatcactgctcaattgcagcattgccaaaataccccagcagaacgcattaggacagagtgtctgtgggacaggtccatagtgcacatacatgacctcccgactgaactccctaggagcatgtgacagtgaaggacagagaggcccagtgtatgctgctgatgataaagcttctgcacaacaaaatctgtcctttctgccccctgcacgggacaagggccagttgtagagagtgcttgtgtcacagggctcctctaggcctctgtgtcctggccacagatgggtgtggaccgcagcctcagggttctcatgacatgacttctttcgttattacatttgtttctctgtctctgtctctgtctctgtctctgtctctgtctctctctctctctctctctctctctctctctctctctctgtgtttatgtgtgtttgtagaggttaaaaggtgctctgtagcatttcttcaaattggtttaaatagtaaaaacgctgagtgagatgtcagataattgggtaaatgttgagacataagagaattaaaggagccaactctatagggacttcttacctgtaccaaatgttcagatggaagtgctggggaggtcctgtctttacaaatcctctatatgaataagcctaaatactgcctcctccagccttatactcctgtctccacctgaggtgcgagccacacgcacccagctcttatatctatcagactggttgaatttcgtgtacctcagtgtggccttgaactcctgatc

SEQ ID NO: 22 - DNA, 1352 bp, Chinese hamster
cttctgagtagtattgcattgagacagcactggatactggaaatcttggggatactgttatgaactgagtgtctctcccctaaagctaagattgaaactaaaatctccaatgtcttgtgctaatagtatttgggtgtggggttttagaatgtctttagaattacatgaaatcatagggaagagaacacttgtgatggaattggcggccttaaatgatgaaaaccatagaccaagcctggaacacttgtcctgtccttttgtaacattcttgtcatgtgctgtcctctgatttcttatgatactgcagaaaggcatttgacagctgctggtgtcatgcttttggacttcccagtttccagagctgtgagccaaatgtatctcttctttataaatctcccagcttatagcattttgtttgtggaaaacaaatagtcttagagaaataattatagattatcagtggccaagatactgatagaagcatcaaagattattttaaaatgccaggccagggagatggttcagagggttaagaggcttgctgccaaggctaatgacctgagttctatcccagaaaccacatgcatagtggaaggatagaaatgactcccggaaagttgtcctttgttctctgcacatgtaccatggcatacacatacatatataaccagtaaggtgtagtaaaagttagagtcaatgcgctattttttatataaataaacataaggacacagcacacgcgcgagcacacatacacacacacacacacacacacacaaaaaaaaaaaaaaaaaatgaaagtagaagagggcctgctgaggaagagggtcccagctggttaggaaggaggatgacaatggtattaaagggtgaaaaatgacccaaattcactatatacttacatgaatctgtcaaatcatttaaaaagccatgtattactgtattagtttcttgtctattgttgtgataaaatgccatgaactaaagcaactttaaaaagtttattttggttttcagttccagaggttcctgagggggcattcataatggtgggagaggcatgtcagctggtagccaaagcaggaagctgagggcctagagagatggctcactagttaagagcactgactcctcttccagaggactcaagttcagttcccagccccacatggcagctcacacctgtctgtagctccagtttcaggggacgcaacacccatggcaaaacattgattaacataaatataaaatgaaaacctccagtttcagggtatccgacacccacgacaaaaaacatcaatgggtataaaaataaaataaaatacttttaaaaagcaggaagctgagagatc

SEQ ID NO: 23 - DNA, 1246 bp, Chinese hamster
ctggtaccttcttttcccagagtctatacaagttaggaaaaacaggaaatgtgggaaaacaggagacagctgaagctcagcatctggcaagacccaacagggtccctctgctaatgatgttccctgagatttgattctaaaacctcagattctttaagtcatgaggtgacatcctcacctcagacttctaaatcacctgtgttctcctttctacaaatgggacaaacatccatccaacattcaagtccaaaacctgagagtcatccttaatttctcttttcctttttagctccctaccgattctttttcaaaaatccaccctttctctcaatcttcacgtcatcagtttttagaaataggtcatttctctccctgagcttatcatctgcctacatgaatctgaactctcattttaaaaatcacatgtagagcttggcccctgccttgagcccgacttctgcctgtccactctgggaactcctgtcctggggactgcaggcaaatcaacttgccccctgaggaccaagcaacctcaagtctgatgacatcactgtgctagtccagttcccacccccacctagagagggagtgccccagacccgcctgaacccaccataagacccatcagagtatcagaccctcttgcatccaccaaagagaaccttggacccatacacaccaggagaggaagagacggcacctgaacccactggaagaagagatgggaagacaacaatataaaaacgcattcaataacagaaaaaacaatatgacaccactagaatctagggactctacgccagcaagacctgaacatcccaacacagatgaagcagaagagaatgacttctgcttgtacttgaagttctatctggggcaatatgacaacaaaaaggagaacaaggggatacaaattggaaaggaagaagtcaaatttttactgtttgcagatgatatgatagttacataagtaacccaaaaaactctaccagggaactactacagctgataaacaccttcagctaagtggaaggatacaagattaactcaaaaaatcactagccctattatacacaggagataaatgggctgagaaataaatcagagaaacatcatcctttacaatagccaaacaacataaaatatcttggggtaatgataaccaaacaagtgaaagacctgtctagcaagaactttgagtcttaaaagaaagaaattaaagaagataccagaaaatggaaagatc